European Patent Specification EP 3 280 257 B1, published June 7, 2023. Title: HUMANIZED T CELL MEDIATED IMMUNE RESPONSES IN NON-HUMAN ANIMALS. Applicant: Regeneron Pharmaceuticals, Inc. The sequence listing filed with the application follows.

SEQUENCE LISTING (91 sequences)

SEQ ID NO: 1 - DNA, 19 bp, Artificial Sequence
  synthetic
cagaacgccaggctgtaac

SEQ ID NO: 2 - DNA, 20 bp, Artificial Sequence
  synthetic
ggagagcagggtcagtcaac

SEQ ID NO: 3 - DNA, 24 bp, Artificial Sequence
  synthetic
caccgccactcacagctccttaca

SEQ ID NO: 4 - DNA, 22 bp, Artificial Sequence
  synthetic
gtgggcaccatcttcatcattc

SEQ ID NO: 5 - DNA, 22 bp, Artificial Sequence
  synthetic
cttcctttccagggtgtgactc

SEQ ID NO: 6 - DNA, 23 bp, Artificial Sequence
  synthetic
aggcctgcgatcaggtggcacct

SEQ ID NO: 7 - DNA, 19 bp, Artificial Sequence
  synthetic
ggtggagaggctattcggc

SEQ ID NO: 8 - DNA, 17 bp, Artificial Sequence
  synthetic
gaacacggcggcatcag

SEQ ID NO: 9 - DNA, 23 bp, Artificial Sequence
  synthetic
tgggcacaacagacaatcggctg

SEQ ID NO: 10 - DNA, 140 bp, Artificial Sequence
  synthetic
tttgtaaacaaagtctacccagagacagatgacagacttcagctccaatgctgattggttcctcacttgggaccaaccctaccggtataacttcgtataaggtatcctatacgaagttatatgcatggcctccgcgccgg

SEQ ID NO: 11 - DNA, 140 bp, Artificial Sequence
  synthetic
cgacctgcagccggcgcgccataacttcgtataaggtatcctatacgaagttatctcgagcacaggcatttgggtgggcagggatggacggtgactgggacaatcgggatggaagagcatagaatgggagttagggaaga

SEQ ID NO: 12 - DNA, 17 bp, Artificial Sequence
  synthetic
cgaggagccccggtaca

SEQ ID NO: 13 - DNA, 20 bp, Artificial Sequence
  synthetic
aagcgcacgaactccttgtt

SEQ ID NO: 14 - DNA, 17 bp, Artificial Sequence
  synthetic
ctctgtcggctatgtgg

SEQ ID NO: 15 - DNA, 22 bp, Artificial Sequence
  synthetic
ggactcccagaatctcctgaga

SEQ ID NO: 16 - DNA, 25 bp, Artificial Sequence
  synthetic
gagtcatgaaccatcactgtgaaga

SEQ ID NO: 17 - DNA, 16 bp, Artificial Sequence
  synthetic
tggtgggttgctggaa

SEQ ID NO: 18 - DNA, 90 bp, Artificial Sequence
  synthetic
ctgtttcttccctaactcccattctatgctcttccatcccgaccgcggcccaatctctctccactacttcctgcctacatgtatgtaggt

SEQ ID NO: 19 - DNA, 80 bp, Artificial Sequence
  synthetic
caaggtttcctcctatgatgcttgtgtgaaactcggggccggccagcatttaacagtacagggatgggagcacagctcac

SEQ ID NO: 20 - DNA, 80 bp, Artificial Sequence
  synthetic
gaaagcagtcttcccagccttcacactcagaggtacaaatccccattttcatattagcgattttaatttattctagcctc

SEQ ID NO: 21 - DNA, 80 bp, Artificial Sequence
  synthetic
tcttccctaactcccattctatgctcttccatcccgaccgcggcccaatctctctccactacttcctgcctacatgtatg

SEQ ID NO: 22 - DNA, 100 bp, Artificial Sequence
  synthetic
gagttcctccatcacttcactgggtagcacagctgtaactgtccagcctgtcctgggctgcaggtggtgggcgttgcgggtggggccggttaaggttcca

SEQ ID NO: 23 - DNA, 100 bp, Artificial Sequence
  synthetic
tcccacatcctattttaatttgctccatgttctcatctccatcagcacagctcgagataacttcgtataatgtatgctatacgaagttatatgcatggcc

SEQ ID NO: 24 - DNA, 100 bp, Artificial Sequence
  synthetic
atacgaagttatgctagtaactataacggtcctaaggtagcgagtggcttacaggtaggtgcgtgaagcttctacaagcacagttgccccctgggaagca

SEQ ID NO: 25 - DNA, 17 bp, Artificial Sequence
  synthetic
tgcggccgatcttagcc

SEQ ID NO: 26 - DNA, 18 bp, Artificial Sequence
  synthetic
ttgaccgattccttgcgg

SEQ ID NO: 27 - DNA, 21 bp, Artificial Sequence
  synthetic
acgagcgggttcggcccattc

SEQ ID NO: 28 - DNA, 18 bp, Artificial Sequence
  synthetic
ccccacagcacgtttcct

SEQ ID NO: 29 - DNA, 23 bp, Artificial Sequence
  synthetic
cgtcccattgaagaaatgacact

SEQ ID NO: 30 - DNA, 15 bp, Artificial Sequence
  synthetic
tggcagcctaagagg

SEQ ID NO: 31 - DNA, 18 bp, Artificial Sequence
  synthetic
ccccacagcacgtttcct

SEQ ID NO: 32 - DNA, 17 bp, Artificial Sequence
  synthetic
acccgctccgtcccatt

SEQ ID NO: 33 - DNA, 18 bp, Artificial Sequence
  synthetic
agcctaagagggagtgtc

SEQ ID NO: 34 - DNA, 20 bp, Artificial Sequence
  synthetic
agaccctggtgatgctggaa

SEQ ID NO: 35 - DNA, 18 bp, Artificial Sequence
  synthetic
cgcttgggtgctccactt

SEQ ID NO: 36 - DNA, 18 bp, Artificial Sequence
  synthetic
tcgaagtggagaggttta

SEQ ID NO: 37 - DNA, 21 bp, Artificial Sequence
  synthetic
tggaatggagtgagcagcttt

SEQ ID NO: 38 - DNA, 20 bp, Artificial Sequence
  synthetic
gcacggtccccttcttagtg

SEQ ID NO: 39 - DNA, 18 bp, Artificial Sequence
  synthetic
tgacttcctaaatttctc

SEQ ID NO: 40 - DNA, 21 bp, Artificial Sequence
  synthetic
ctggcggcttgaagaatttgg

SEQ ID NO: 41 - DNA, 24 bp, Artificial Sequence
  synthetic
catgatttccaggttggctttgtc

SEQ ID NO: 42 - DNA, 26 bp, Artificial Sequence
  synthetic
cgatttgccagctttgaggctcaagg

SEQ ID NO: 43 - DNA, 21 bp, Artificial Sequence
  synthetic
cctcacttgggaccaacccta

SEQ ID NO: 44 - DNA, 20 bp, Artificial Sequence
  synthetic
ttgtcccagtcaccgtccat

SEQ ID NO: 45 - DNA, 24 bp, Artificial Sequence
  synthetic
tgcatctcgagcacaggcatttgg

SEQ ID NO: 46 - DNA, 100 bp, Artificial Sequence
  synthetic
atggagtagtcagaacacactcttcagaagggactcctgatttcaaagggggtaccgggccccccctcgaggtcgacataacttcgtatagcatacatta

SEQ ID NO: 47 - DNA, 108 bp, Artificial Sequence
  synthetic
ggccatgcatataacttcgtatagcatacattatacgaagttataccggtgcgatcgcgcgcttccctcttctaaccactaattcaaaaaggattgtaagtaatgttt

SEQ ID NO: 48 - DNA, 145 bp, Artificial Sequence
  synthetic
agacagacccctaaacacctccaaattaaaagcggcaaagagataaggttggagctccaccgcggtggcggccgccaccgcggtggagctcgaggtttccggtacttaacaacagagcacagatttagtggtgagggactctctc

SEQ ID NO: 49 - DNA, 100 bp, Artificial Sequence; identical to SEQ ID NO: 46
  synthetic

SEQ ID NO: 50 - DNA, 109 bp, Artificial Sequence
  synthetic
ggccatgcatataacttcgtatagcatacattatacgaagttataccggtgcgatcgctcaagcatgcaagggtaacatatgttatgagattatattttctttatctca

SEQ ID NO: 51 - DNA, 100 bp, Artificial Sequence
  synthetic
atggagtagtcagaacacactcttcagaagggactcctgatttcaaaggggggtaccgggccccccctcgagaagttcctattccgaagttcctattctc

SEQ ID NO: 52 - DNA, 108 bp, Artificial Sequence
  synthetic
gttcctattccgaagttcctattctctagaaagtataggaacttcctagggcgatcgctcctctccaggctcgaattagtattacagttgaggcacgttgtcctcccg

SEQ ID NO: 53 - DNA, 100 bp, Artificial Sequence; identical to SEQ ID NO: 46
  synthetic

SEQ ID NO: 54 - DNA, 108 bp, Artificial Sequence
  synthetic
ggccatgcatataacttcgtatagcatacattatacgaagttataccggtgcgatcgccgcctccatttccttcataggaaacatgaagtgaatggggctgtgtgtgt

SEQ ID NO: 55 - DNA, 100 bp, Artificial Sequence; identical to SEQ ID NO: 46
  synthetic

SEQ ID NO: 56 - DNA, 108 bp, Artificial Sequence
  synthetic
ggccatgcatataacttcgtatagcatacattatacgaagttataccggtgcgatcgctgggagcacgttccattattataacaactttctgaacacaagagggcagt

SEQ ID NO: 57 - DNA, 100 bp, Artificial Sequence; identical to SEQ ID NO: 46
  synthetic

SEQ ID NO: 58 - DNA, 108 bp, Artificial Sequence
  synthetic
ggccatgcatataacttcgtatagcatacattatacgaagttataccggtgcgatcgctttaaggtgaggaggcaggcaataccccctctccaccgcattctcaatcc

SEQ ID NO: 59 - DNA, 100 bp, Artificial Sequence
  synthetic
gggggggtggggtggaggaggagggtacagcatctcctctccttcctctctggtaccgaagttcctattccgaagttcctattctctagaaagtatagga

SEQ ID NO: 60 - DNA, 108 bp, Artificial Sequence
  synthetic
gaagttcctattctctagaaagtataggaacttcctagggtttcaccggtgcgatcgcgtgaatatactaaaaaccacttaattatatatttgaaagggtggatgtta

SEQ ID NO: 61 - DNA, 108 bp, Artificial Sequence
  synthetic
ctctctcctacccagctcctctcacacgagcctgaaggccctgccaaggtggcgcgcctttcaaattgttgttgagttcaaagtgggcaacagaaaagggggtgtgag

SEQ ID NO: 62 - DNA, 130 bp, Artificial Sequence
  synthetic
aataaatagtaaatttctgtagaatcataatgaggtctagacccccgggctcgataactataacggtcctaaggtagcgaaatggcgcgtaatcaagcccagctcttcatgctgcatttttatcttcttt

SEQ ID NO: 63 - DNA, 100 bp, Artificial Sequence
  synthetic
ttgactcgggggtgcctgggtttgactgcaatgatcagttgctgggaaggaccggtataacttcgtataatgtatgctatacgaagttatatgcatggcc

SEQ ID NO: 64 - DNA, 100 bp, Artificial Sequence
  synthetic
ccggcgcgccataacttcgtataatgtatgctatacgaagttatgtcgacataaggtaagacagagtcgtcccttcccatctggaaccctctacctttct

SEQ ID NO: 65 - DNA, 107 bp, Artificial Sequence
  synthetic
gttgatgaatcataaaagaagagatattcaagaaaaggatggccacactgcggccgcagaggtattcaaggaaaatgcagactcttcacgtaagagggatgaggggc

SEQ ID NO: 66 - DNA, 100 bp, Artificial Sequence
  synthetic
tccccggagtcggagggtggaccggagctggaggagctgccgcggtggcggccgatgccatttcattacctctttctccgcacccgacatagataaagct

SEQ ID NO: 67 - DNA, 100 bp, Artificial Sequence; identical to SEQ ID NO: 59
  synthetic

SEQ ID NO: 68 - DNA, 108 bp, Artificial Sequence
  synthetic
gaagttcctattctctagaaagtataggaacttcctagggtttcaccggtgcgatcgcgaagcaattaactgcccctggtccagttgcctcctctgataatgcattgt

SEQ ID NO: 69 - DNA, 100 bp, Artificial Sequence; identical to SEQ ID NO: 59
  synthetic

SEQ ID NO: 70 - DNA, 108 bp, Artificial Sequence
  synthetic
gaagttcctattctctagaaagtataggaacttcctagggtttcaccggtgcgatcgcgttatctagtagacttaattaaggatcgatccggcgcgccaatagtcatg

SEQ ID NO: 71 - DNA, 100 bp, Artificial Sequence
  synthetic
gttttccagacttcaacttgactatcagccagaaattcagtggcaaacccccacccagtccctaagtgaaggcccctggggagtatggttagggctcagg

SEQ ID NO: 72 - DNA, 100 bp, Artificial Sequence
  synthetic
cacccaccaaagaaagtgcccaggagaagggcaaggagagagcagagcatagttcaagatggtctttgtctaggcttgtctactctgcacttgtacttcc

SEQ ID NO: 73 - DNA, 202 bp, Artificial Sequence
  synthetic
aggggaaacccgcaaaggatgggacatagggagacagctgttaacatctgaaacatgaccttcttttctgtgcagcacaactcctagctgtcactcaagggaagaaagtggtgctgggcaaaaaaggggatacagtggaactgacctgtacagcttcccagaagaagagcatacaattccactggaaaaactccaaccagat

SEQ ID NO: 74 - DNA, 240 bp, Artificial Sequence
  synthetic
ctggtcacctggatgaagtgagggagggccctctgggtttggggctggttttgaactgagacatccatgagccagcctggggctggcttcactgaagatcatctatgtcgggtgcggagaaagaggtaatgaaatggcacatgctatgtacaaactctattgctgagcagcacccagtcctgagctggctctgaattgagggtgaaattcacacattctcccccaacatctataatctgg

SEQ ID NO: 75 - DNA, 151 bp, Artificial Sequence
  synthetic
tatggagtgaaagcctttggtgtctgagatctggtcttagttaaactctgggatcggcgcgccgaattcctgcagcccgggctcgagataacttcgtataatgtatgctatacgaagttatatgcatccgggtaggggaggcgcttttccc

SEQ ID NO: 76 - DNA, 151 bp, Artificial Sequence
  synthetic
agtattgttttgccaagttctaattccatcagacctcgacctgcagccctagataacttcgtataatgtatgctatacgaagttatcctaggccagagggcttgggttgacagaaactcagtggcattcttatccagagtttctctacacc

SEQ ID NO: 77 - DNA, 18263 bp, Artificial Sequence
  synthetic
  misc_feature (2957)..(2957): n = A,T,C or G
  misc_feature (3193)..(3193): n = A,T,C or G
aagaaagtggtgctgggcaaaaaaggggatacagtggaactgacctgtacagcttcccagaagaagagcatacaattccactggaaaaactccaaccagataaagattctgggaaatcagggctccttcttaactaaaggtagggttgcctggctccccatccagggaggaaaacacactatggagtgaaagcctttggtgtctgagatctggtcttagttaaactctgggatcggcgcgccgaattcctgcagcccgggctcgagataacttcgtataatgtatgctatacgaagttatatgcatccgggtaggggaggcgcttttcccaaggcagtctggagcatgcgctttagcagccccgctgggcacttggcgctacacaagtggcctctggcctcgcacacattccacatccaccggtaggcgccaaccggctccgttctttggtggccccttcgcgccaccttctactcctcccctagtcaggaagttcccccccgccccgcagctcgcgtcgtgcaggacgtgacaaatggaagtagcacgtctcactagtctcgtgcagatggacagcaccgctgagcaatggaagcgggtaggcctttggggcagcggccaatagcagctttgctccttcgctttctgggctcagaggctgggaaggggtgggtccgggggcgggctcaggggcgggctcaggggcggggcgggcgcccgaaggtcctccggaggcccggcattctgcacgcttcaaaagcgcacgtctgccgcgctgttctcctcttcctcatctccgggcctttcgacctgcagccaattgttgacaattaatcatcggcatagtatatcggcatagtataatacgacaaggtgaggaactaaaccatgggatcggccattgaacaagatggattgcacgcaggttctccggccgcttgggtggagaggctattcggctatgactgggcacaacagacaatcggctgctctgatgccgccgtgttccggctgtcagcgcaggggcgcccggttctttttgtcaagaccgacctgtccggtgccctgaatgaactgcaggacgaggcagcgcggctatcgtggctggccacgacgggcgttccttgcgcagctgtgctcgacgttgtcactgaagcgggaagggactggctgctattgggcgaagtgccggggcaggatctcctgtcatctcaccttgctcctgccgagaaagtatccatcatggctgatgcaatgcggcggctgcatacgcttgatccggctacctgcccattcgaccaccaagcgaaacatcgcatcgagcgagcacgtactcggatggaagccggtcttgtcgatcaggatgatctggacgaagagcatcaggggctcgcgccagccgaactgttcgccaggctcaaggcgcgcatgcccgacggcgatgatctcgtcgtgacccatggcgatgcctgcttgccgaatatcatggtggaaaatggccgcttttctggattcatcgactgtggccggctgggtgtggcggaccgctatcaggacatagcgttggctacccgtgatattgctgaagagcttggcggcgaatgggctgaccgcttcctcgtgctttacggtatcgccgctcccgattcgcagcgcatcgccttctatcgccttcttgacgagttcttctgaggggatccgctgtaagtctgcagaaattgatgatctattaaacaataaagatgtccactaaaatggaagtttttcctgtcatactttgttaagaagggtgagaacagagtacctacattttgaatggaaggattggagctacgggggtgggggtggggtgggattagataaatgcctgctctttactgaaggctctttactattgctttatgataatgtttcatagttggatatcataatttaaacaagcaaaaccaaattaagggccagctcattcctcccactcatgatctatagatctatagatctctcgtgggatcattgtttttctcttgattcccactttgtggttctaagtactgtggtttccaaatgtgtcagtttcatagcctgaagaacgagatcagcagcctctgttccacatacacttcattctcagtattgttttgccaagttctaattccatcagacctcgacctgcagccctagataacttcgtataatgtatgctatacgaagttatcctaggccagagggcttgggttgacagaaactcagtggcattcttatccagagtttctctacaccaactgctggtggcccagggaaaggtggtatgtgaatttcaatattttaatatttaatattcatgaacttattttagtgagttttagaacaatcactatcacttaaaacccgtgatttcttgagtattgttgctacagacctatgtagataatactttgcacagtgactcatatgtataatcctagcactgtgggaggctgaggccggaggattgcttgagtccaggagttcaagaccagcctgaacaacatagtgagactctgtctctatgaaaaaaaatatatatatattttttttggagacaaggtctagttctatcacccaggctccagtgcagtggtgtgatctcggctcactgcaatctccacctcccaggctcaagtcatcatcccacctcagcctcccaagtagctgggactacaggcatgcaccaccatgccaggctaatttttgtattttttatagagacagggtttcaccatgttggccaggctggtctcgaactcatgagctcaagtgatccactcaccttggcctctcagagtgctggaattacaggtgtgtgtcactatgcctagccaaaaaaaatttttttaattaaaaaaaaaaaggccggctgtagtggctcacacctgtaatccagaactttgggagtttgaggtgggcagatcaccggnggtcaggagttcaagaccagtctggccaacatggtgaaacccggtctctactaaaaatacaaaaattagccaggtgtgggggtgcagtcctgtacttccagctactcaggaggctgaggcaggagactcgcttgaacctgggaggcaaaggctgcagtgagctgagattgcaccactgcactccagcctgggtgacagagcaagacttcatctcaaaaaaaaaaaaaaagctgcanatttattattattattattagtttatttatttatttttttgagacagagtctcgttctgtcgcccaggctggagtgcggtggcgtgatcttggctcattgcaacctccacctcccgggttcaagtgattctcctgcctcagcctcccgagtagctgggactacaggcgtatgccaccatgcctggctaattttttgtacttttagtagagacagagtttcacggtgttagccaggctggtcttgatctcctgacctcgtgatttaccctccttggcctcccaaagtgctgggattacaggcgtgagtcactgtgcccggcccagaatcatttttttctacttttttttttttgaggcaaactctcgatctgttgcccaggctggagtgcagtgggcatgatcttggctcactgcaagctctgcctcccaggttcaagcaattctcctgcctcagcctcctgagtagctgggactacaggcgtgtgccaccatgcccggctaatttgcgtatttttagtagagaccggttttcatcatattggccaggctggtcttgaactcctgacctcaagtgattctcccaccttagcctcccaaagtgctgggattacaggcatgagctactgcacttggccttttctcctggttttaaaactattatatgctcattacaaaatatttggtcaatgaagaaaagaatatggaagaaaatcaaatgcatgcatacttctatcactcagagatatcctctgctaacattttgattgattttcttccaatctttttttttttttttctttttgagacagggtctcactctgctgcccaggctggagtacagtggcatgaccacaacacatcacagcctcaagtgatcttcccacttcagccttcccagtagctgggactacaggtgcacgccaccatgttcacctaattttttactttttgtagagatgagacttcaccatgttgctcaggctggtcttgaattcctaggctcaagtgatcttcccgctttggcctcccaaagtgctgggattataggtatgagccactgcatgtggcctattttcttccactgttgttcggcgtggagaatattatatacataattacgtaaatgatatcatactgtatataccttttttcctactccttccttaagttatatcataatgagactaccaattattagactttttttcttttttttgagacggagtctcggtctgtcacctaggctggagtgcaatggcgcgatctcagctcgctgcaacctctgcctcccaggttcaagcaattctgcctcagcctcccgagtagctgggactacagacacgtgccaccatgcccagctaacttttttatttttttattagagacagggttccaccatgctagcaggatggtctcaatctctcgacttcgtgatcagcccggcttggcctcccaaagtgctgggagtacaggtgtgagccaccgcactcggcctagactaactatttaaagtaatctggcaatgtttaacgaatacaaaactctaaaacccttggacctaataatagctattttggaaagtctacttgacagaaataaaattgtgaatattcttttttgttgtttttttgagacagagtctcatttggacgcctaggctggagtgcagtggcatgatctcggctaactgcaacctccacctcctgggttcaagtgattctcctgcctcagcctcctgagcagctgggattacaggtgtgcaccaccatgtctggctaatttttgcatttttagtagatggggtttcaccatgttgaccagggtggtctggaacttctaccctcaagtgatctacccaccttggcctcccaaagtgctgggattacaggtgtgagccaccacgcctgaccagtgaacacttaataatatctatggaaaggtgttattataagaattgcttgtggggccgggcgtggtggctcacgcctgtaatcccagcactttgggaggctgtggcaggcggatcacgaggtcaggagatcaagatcatcctggctaacacggtgaaaccccgtctctactaaaaataccaaaaaattagccaggcgtggtggcgggcacttgtaatcccagctatccaggaggctgaggcaggagaattgcgtgaacccaggaggcggaggtcgcagtgagctgagaccgtgccattgcactccagcctgagtgacagagtgagactccatcacaaaaaataaataaataaataaataaaatataaataagtaaataaaggtcaggagtggtggctcacgcctgtaatcccagcactttgggaggccgaggtggacagatcatgaggtcatgagatcaagaccatcctggctaacacagtgaaaccctgcctctactaaaaatacaaaaagtcatccaggtgtggtggcacacacctatagtcccagctacttgggaggctgaggcaggagaatcacttgaacccaggaggcagaggttgcagtgagctgagatcgcgccactacactccagcctaggcgacagagcaagactctgtctcaaaataaataaataaataaataaataaataaataaataaataaaataaaaagcacacacacacacacacacacacacacacaatgcaaaagacccaccctactacaactaacattatatttaatggtgaaaaactgaattctttctccctaagtgcaggaataagacaaagatgtctgctcttactactcttattcaacataatactgcaatcccttgccagtgcaataaggcaagaaaaatgaaataaaaggaaaactgatcagaaagaaagaaataaaactgttcctatttgtggatgacatgattacatagaaaatctcaaagaatctgtaagaaacttcttagaattaataaatgaattcatcaaggttgcagaatataagataaacataaaaaatctattgtatttctatatattagcaaggaacatgtgtacacagaaattaaaactacaataccatttataattgctcaaaaaggccaggcatggtggctcacacctgtaattcctgcactttgggaggccaaggtgggaagattgcttaagcccaggagttcaagaccagcccgggcaacatagtgagaccttgtctctacaaaaagtaaaaaattagctgagcatggccgggtgcagtggctcactcctgtaaccccaacactttgggaggctgaggcgggcggatcatgaggtcaggagatcgagaccatcctggctaacacggtgaaaccctgtctctactaaaaacacaaaaaattagctggatgtggtggcaggcgcctgtagacccagctactcgggaagctgaggcaggagaatggcgtgaacctgggaggcggagcttgcagtgagctgagattgtgccactgcactccagcctgggtgacacagtgagactacgtctcaaaaaaaaaaaaaaaaaaattagctgagcattatggtgtatgcctgtagtcccagctactggggaggctgaggtgggaggattgcttgagccctaggagggcaaggctgcagtgagccatgatcacaccactgctttccagcctcggtaggagagcaagaccctatctcaaaaaaaaaaaaaaaaaaaaaagaaaagaaaagaaaagaaaagaaaaagaaagagagaaagaaatacttaggtgtaaatctaaaaaacatgcgtagggccaggtgcagtggctcatgcctgtaatcccagcactttgggaagttgaggctggcggatcacttgaagtcgggagtttgagaccagcctggccaacatggtgaaaccccgtctctactaaaaatgcaaaaattaggcaggtgttgtggcgcatgcctgatcccagctactttggaggctgaggcaggagaattgcttcaacccgggaggcagaggttgcagtgagccaagactgttccactgcactccagcctgggcaacagagtaagagtctgtctcccgaaaaaaaaaaaaagaaaaaagaaagcattgaattgtatgctaaaaactacacgatgctgattaaagaagtcaaagaagatctaaatatatggagagacatgctgtactcatggattgatggattggaagactcaacataagacagatatcaattttccccaaattaatatacaagtttaatccaattcctataaaaataccagcaagattttttgtagatataaacaagttggccaggtgtagtggcttacacctgtaatcctagcactttgggaggctgaggtgggaagatcgcttgagcccaggtgttcacgactgcagtgagctatgattgtgtcactgcattccagctggcactccagcctaagtgacaaagggagaccctgtctcaaaaacaaaaacaaaaccaaaataattttgctctgcaaaatccctattaagaagaagaaaagaggctgggcacagtggctcaccgctgtaatcccagcacgttgggaggctgaggcaggctgatcacttcagcccagaagtttgagatcagcctgggcaacatgaggaaaccccgtctctaccaaaaaaaaaaaaaggtacatacacacacacacacacacacacacacatacacaagtatatacacatatatatacacatacaggtgaatagatgtatatacatctatttattgtgaatatacatctatacacacacgtgtgtgtacacatatatttaaaatttatttttatttatttatttatttttgagacagagtcttgctctgtcacccaggctgggtgcacctgtattcccaacgacacaggaggctgaggtgggagaatcactgagccagggaggcagaggttgcagtgagccaagatgttgcctggttgcctgggcaacagagcgagaccctatatcaaaaaagaagaataataagaaaagacagtttacagaatataagaaaatatattcacaatccacatacttagcaaaggactggtatctagaatatgataaacaactctcaaaactcaaaaccaaaaaaatgaacaattcaattagaaaacaggccgaaaaggacatacagttggcaaataagcacatgaaaagttgttcaacatcattaatcattagggatatgtacattaaaaccacaataggctatcactaaacctatcagaatggctaaatacaaaattggaacaccaccaaatgctgatgaggatgtggagaaactgggtcattcttccaatattggtgggaggctaaaatggcaaagccactctggaaaacagtttgatagtttcttataaaacaaaacatgcggccgggcgcggtagctcacgcctgtaatcccagcactttgggaggccgaggcgggtggatcacgaggtcaggagatcgagaccatcctggctaacacggtgaaaccctgtctctactaaaaatacaaaaaattagccgggcgtggtggcgggcgcctgtagtcccagctactcgggaggctgaggcaggagaatggtgtgaacccgggaggcggagcttgcagtgagccgagatcgcgccattgcactccaacctgggagacggagggagactccgtctcaaaaaaacaaaaacaaacaaacaaaaaacatgcaacaatccagcaatattgcacccctaggcatttatcctagagcaatgaagacttatgcccacacaaaaagctgcacacaaatgttcatagcagctttattcatggtagccaacaattagaaacaatctagatgtccttcaactggtgaatgattacatccataccacgaaatacttttcagcaataaaaaggatgaatcatagtacacaccacaacctggatgaatctccagggaattatgctgagtgaaaaaaagccaatctcaaaaggtaatatactgtattaatccatttatataacattcttaaaataactaattatagaaatggagaacagatgagtgattgccaggggttaaggggctcagggatggggaggggaaggggtatggctacaaaaagcaacaaccttatggcgccggaaatgttctgtattctgattgtgtcaatgtgagcatactggttgagatatagtgctacagttttgcaagttattaccatcagagtaaactggatagagggcacataggatttctctgtattacttcttacaactgcaagtgaatctacaattatctcaaaataataagtttagtttaatgctaggcgtggtggctcacatctgtaatctcagctctttgggaggctgagacgggtggatggcttgagtccaggagttcgagaccagcctggccaacatggcaaaaccggtctctactaaaaatacaaaaattagctgggcgtggtggcaagtgcctgtagtcccagctactcgggaggctgaggcaggagaattgcttgaacccgggaggtggaggttgcagtgagccgagatcacgccactacactgtagcttgggcgacagagtgaggctctttctcaaaaaaaaaaaaaaaaaaaaaaaagcaggcaggcagggccaggaaagcgtataatttttgtagttcaaatgactaacctaaaaagtgaagattggccaggcgcagtggctcacgcctgtaatcccagcactttgggaggccaaggcgggtggatcacgaggtcaggagattgagccactctggctaacacagtgaaaccccgtctctactaaaatacaaaaaattagctgggcgtggtggcacccgcctgtagttgcagctacttgggaggctgaggcaggagaatcacttgaacccaggaggcgaagttgcagcgagccgagatcacactactgcactccagcctgggtgacaaagtgagattctgtctcaaaaaaaaaaaaaaaaaaaaaaaaaaaaaaaagtgaagtttacctttttttttaaatttttcttcttttccttccctactttgtgagataattttcttctttttaaaaagccaagagcttacttctgtaagtaaagattatcttaagacaacttagaaatgtatattattagtattttctatttcattgtaagttatttgtaaatattggttttggtgctaacctagaattccatcaaattaattgtcccctaatatatggccattatcattttgtctaacattgtatcctattaacaatgctgtaagtattatttttgtagctaaattatggtttgcattttaaaattattgttttaaggataaagttccagaaatgaaattaaggatatgaactttttgagcacatcttgtcagcactgagtagtattatttaaaacttttggggggggcaattttataattgaaaaatatatcattgttttaatttgcatttctttcactgcctatgagattaaaacaatgcactactttccaaaaattcttaagtcttttgtgttgatgcttttgttctgtttctatggatctcatcttccttcagaacagctccccttcccaacttcctgatttctaacaataacagtatcaccctccttgttctcccaatttctgaaacacagagtcatgtttttttctctgcttcaatccctggtttcctatcgtcatcaattatgacctttccttgctttgaaagtgttttgggccgggcatgatgtctgccacctattgtaatcctagcactttgggaggctgaggcggctggatgacttgacctgaggatttcgagaccagcctgggcaacagggcgaaacctcgtctctacaaaaaatacaaaagttagtcgggagtggtggcacatgcttgtagtcccagttacttggggggctgaggtggcaggatctcttgagcccacgaggtagatgttgcagtgagccgtgattgcgccactgcaccccagcctaggtgacagagtgagaccctgtctcaaaaaaaaaaaaatgttctagtttcttcctcttctttgttcccatgggaatgccaccatcaccagccaaggctcacatacctcccacctggattacagtgagcttccaggtaatttggtctgctactagtctcgcctacttggatttcccttccccctgctgcagcattgccttccaaagccatgctttgcacatgccacatcctagcccattagactaagcctagaagcctctgcaggacgttcaccctctcagcgccactgctcagtttcccagtggaaacctctgcacccaggaggtttccccacagcttgcctgtgctgcctctctggagcttttctcccttcctgtaatgtccttgctgctccccgtctctagtccattgcctatacctctttttttttttttttttgagatggagtctctctctctcatccaggctggagtgcagtggcgcgatctcggctcactgcaacctttgtctcctgggttcaagggattctcctgcctcagcctcccgagtaactgggattacaggcgtgcaccaccattcctggctaatttttgtatttttagtaaagactgggtttcaccatgttggccaggctggtcttgaactcctgccctcaggtgatccacctgcctcggcctcccagagtgctgggattacaggcgtgagccaccgcacctgccacaggcccatacctcttttaagtcttcattcaataccagttgtcccatgaatttgtcccagactcactcatatgcttagacctttcatattatcttgccatagctttttcaaagtatgggacagcatggacaagcaggccatggttttcttttgaagagaagcaaggaggcagagttattttaggaggagggttatacatttcattttgaaccaattgcgtttggggtgatggcaggatattaacataaacttatttcttggaccattggaaatgtgtgcctagaactgaggagagaggtcagggctggcagtaacaacttggccacaatctgcagagctgactggggatgaggtggaatttagaatgtctgtagaaacggggaagagaaccaaagacagagtctgggacaacacctaaatgtagatgtcagagcaagagttcaagacgaagaaaaacgaatcatacttagaaatggaggggaggaacaaaagaggcggagcaaagtggggcagaaccagagtaggccacgcttttaagaagtttggtaaaggaactgtgaaaggaatgtagttgaatttcagggtaagctggggaattaaagcagtgtgtagatccagggcaaacagcaagtagggcaggaaccactgaaggaacaaataaagggggaggttgggtccaggttgtcttgagtagggaagtttttttaaaaagtgtgaaactgaaggtgtggggtggattgggtgcctgccgtgctctgaggaagcttggggcaactgtgtgctgaggctgtgaggttgtctggaaggggctcctggacagtaagagctgagcagtggggaagaggactgtgtggtctggaagaggagagaaaggagagtgagtgactgaactggtatccaggctcccacaccaaggcagaaagagggagaggacctgggcatctcagggaggcagaggcagtaccaagcagggtgagaggctttagtcttagccacctttgccccattcctccaaatatacattctaagtaaaaacaaaacaaaacagaactgtttgctatgtaaatttagcttctaaagccctgttctacagagattttggagcttccactgcacccagaaaatgcacagctaaagagaaaacttcccttggtgatggttattagattttacaagaagaggccaaaggagacacatacttatgccagaagaactttccagagatagcattgcatagcgaaatagcctgaattatttttattttttaaaacattttttcttttcttttttcttttctttttctttttttttttttttttttgagacagagtctcactctgtcacccaggctggagtgcagtggcgtgatcttggctcactgcaatctccacctcccgggttcaagccattctcctccctcagcctcccaagtagctgggattacaggcatgcgtcactatgctctggctaattttttttttctttttttttttggtatttttagtagagatggggtttcaccatgttggccaggctggtcttgaactcctgacctcaagtgatccaccgccttggcctcccaaagtgctgggatttcaggcgtgagccaccgcacccggccaaaaatttcttttctttaagatgaggcctcactctgttgcccaggctggagtgcagtgttacaatcatagctcactgtaactttgaactcctgggctcaagtgatcctcctgcttcagcctctcaagtagctgggattacaggcatgtgccaccacacccagctaattttttttaaaataattttttttagagacgagggtctcgattggctgcctaggttggtcccagactcctgacgggctgcattttaatcctagctccaccacttacgggagtcaaaattcaaaagatagaaaagggcatataggctgggtgcagtggctcacacctgcaatcccagcaatttgggaggctgaggtgggcgggttgcttgaggtcaggagttcgagatcagcctgggcaacatggcaaaacttgtatctactaaaaatacaaaaattagccagatgtggtggtgtacacctgtaatcccagctactccgaaggctgaggcaagagaatcccttgaactcaggaggcagaggttacaatgagcagagatcgaacactcgactccataaaaacaaacaaacaaaaaaagaaagcaggctgggtgtggtggctcacgcctgtaaccccagcacttcgggaggccaaggcgagcggatcacctgaggttgggcattcgagaccagcctgaccaacaaggagaaaccctgtctctactgaaaatacaaaattagccgggcttggttgcgcatgcctgtaatctcagctactcgggaggcagaggcaagataattgcttgaacccgggaggcggaggttgcggtgagccaagatcatgccattgcactccaacctgggcaacaatagcgaaactccatctcaaaaaaaaaaaagcaaagggcatatagtgaaaagctttcttcctacacatgagtattcacttcctcttcctagaggcaaccaaggttatttttgtgtgtgtgtgtgtgtgtgtgtgtgtgtgtgtgtgttttgggacagtctcactctctcaccaaggctggaatgcagtggtgcgatctcactgcaaactctgcctcccagtctcaagcgatcttgtgcctcagcctcccagtttttttttcttttaaatggggtctcattctgtcgcccagggtggagtgcagtggcatgatcatagctcactgcagcctcgacctcctgggtcaggttatcctcccacctcagcctccggcatagctggggctactggcatgcaccaccacactcagttaattttttttcttttttgagacagagtctcactctgtcacctagactggagtgcagtggtgccatctcatttgtttcactgcaacctttgacttctgggctcaagtgattctcccacctcagcctcccaaggcggctaattaaaaaaaatttttttttttttttttttagagatggggtttcgccatgttgcccaggctgatctcgaactcctgggcacaaacaatctttccacctcgatctttcaaagagctgggatgagagatttccaccatgcctggcctcattttcttttttaatttttttttagacattatagctctttttaatggcctcattttcttatgtttaattcgagaattattcttttcatatacaaagaatatattttctccacctttaaaaacaaatagtagactgtttaacatctcgctttattcagttagtgatgtttcttagatacgggtccaaattagtacacaaagcacttcctcattcctctcttacggctgcatagcagtccactgaatgggtgagctatgatctatttaacctattctttattgatggacatttggttttgtatatacatttgtaattctgtatagattacaaatcaccatccaaagaaattgtactggtttattctcctacaatgtgtgagagttgggtaattacttaatctcaatatgtgagagtttaggcagttacctaatctctctgagtctcagtttctctatctgcaaaataaacaaaacagtgttgacagtatctatttctcggaattattgtggagattactgagatgatgcctgtaaagtatttggcatgtaggagttggtgctctccaaataaggatatgattttatttgtatttgtgagctactgtcccagccaggtaaatggatatgatgagacctccttgccagaccgggtttctctgattagaacgaggagcagatgttgcaggaaattagcaactgatatcagaagagccgtgggcattctcttgccagaggtgccctgtctccagggcgcctcagtccccccccatatgtcttctgctcccaggtccatccaagctgaatgatcgcgctgactcaagaagaagcctttgggaccaaggaaactttcccctgatcatcaagaatcttaagatagaagactcagatacttacatctgtgaagtggaggaccagaaggaggaggtgcaattgctagtgttcggatgtgagtggggcaggtggggatgaggatacctcctgcctggttcccttccccactactcccacccctgcaccaaatccagcctgagctggtgataccgcagcagccccaagaggaccaggctgtcaaactggcctccaaatgtcttaaaacccttcttgatcaggtgagggatgctggtgggcggaggagggaagaggccttgggaaaaggaaagaaaagggaaggaggcaagggaaggagggagagagactggggaagagaggatgaggggagaggaggaaagaagagagagaggaggggagagggaaaccctatcttggctgggggtgcgcagctgggtgctgggaggaaggagatgttgggacggcgataatggagagatgttgttggtttcctgttgtctgcccttctccttggggatggtatgtgtgtgacacagctggcctttccctccacagtgactgccaactctgacacccacctgcttcaggggcagagcctgaccctgaccttggagagcccccctggtagtagcccctcagtgcaatgtaggagtccaaggggtaaaaacatacagggggggaagaccctctccgtgtctcagctggagctccaggatagtggcacctggacatgcactgtcttgcagaaccagaagaaggtggagttcaaaatagacatcgtggtgctaggtaagggaagcccctcttcgcgcagtctcctccctgccccaggggctgacagcccctccctctgctctgactgccctgtttctggttctggtgctgggaggtcaggagtggagaagactaggtcccctagagctgaggcctgtcttgaaggactcactggggccctcatcctcagggggctgattggcagccacccctcagtgtggtggacatggagaaaggaaaggctggggaaggtaaggatgctagaggcccgagtctcctttggaggccccaaaggaggaatgtcagggagcttactttctttgttgcctcagctccacacccctaccaagttggcaaatccacttactcagggacactaacaccagtaagccaaccctgatgatgttctatgttgtacctctggacctctaagccaggccactgtggggagaccaaggtcctaccccagatcctgtcccctgggtgcttatgtgacttaaggtagacataaggtagtgtgccagtttagtgcatgtacgctgattgaaatcctggttctgccacaaccatgtgaccttgggtgagttactaaacctctctgcaccttggtttcagcctctgtgaaatggggatgatgttaactgccatagtgactacctcgtattaagttgaggactgatatacgtaaggcactgaaaatggtgcctggcacagagtaagccctagttaagtgttcgctgttattttgtgaagggtgatgaatacgcctctaaggagtggaggccaaatggcttctgtggtccaggaatcctaaggacagcaaggatcccctgtggctgggctgctctgtgatggcttccgggaggagggaggtggcctgctgtaggaaaatgctgggtggaagaagggagagaaggctggagaggtaggaaggaactgaagtatctgaagtgacaaggtgggtgtctggactcgtcgggtccccttccatctccctgctgcctccacatgccaaccccactcgtgcaccctcatcttcctatctcctcacccagggtctctcccttcccacctccagctttccagaaggcctccagcatagtctataagaaagagggggaacaggtggagttctccttcccactcgcctttacagttgaaaagctgacgggcagtggcgagctgtggtggcaggcggagagggcttcctcctccaagtcttggatcacctttgacctgaagaacaaggaagtgtctgtaaaacgggttacccaggaccctaagctccagatgggcaagaagctcccgctccacctcaccctgccccaggccttgcctcagtatgctggctctggaaacctcaccctggcccttgaagcgaaaacaggaaagttgcatcaggaagtgaacctggtggtgatgagaggtgaggggccaggccagggaggggtgggcaggggaaggagttggaggggcctggcccagggctccctctgaggcaagccaggccccaagaggggatgcctaggccctggtcacctggatgaagtgagggagggccctctgggtttggggctggttttgaactgagacatccatgagccagcctggggctggcttcactgaagatc

SEQ ID NO: 78 - protein, 458 aa, Artificial Sequence
  synthetic
MCRAISLRRLLLLLLQLSQLLAVTQGKKVVLGKKGDTVELTCTASQKKSIQFHWKNSNQIKILGNQGSFLTKGPSKLNDRADSRRSLWDQGNFPLIIKNLKIEDSDTYICEVEDQKEEVQLLVFGLTANSDTHLLQGQSLTLTLESPPGSSPSVQCRSPRGKNIQGGKTLSVSQLELQDSGTWTCTVLQNQKKVEFKIDIVVLAFQKASSIVYKKEGEQVEFSFPLAFTVEKLTGSGELWWQAERASSSKSWITFDLKNKEVSVKRVTQDPKLQMGKKLPLHLTLPQALPQYAGSGNLTLALEAKTGKLHQEVNLVVMRVAQLNNTLTCEVMGPTSPKMRLTLKQENQEARVSEEQKVVQVVAPETGLWQCLLSEGDKVKMDSRIQVLSRGVNQTVFLACVLGGSFGFLGFLGLCILCCVRCRHQQRQAARMSQIKRLLSEKKTCQCPHRMQKSHNLI

SEQ ID NO: 79 - protein, 293 aa, Artificial Sequence
  synthetic
KKVVLGKKGDTVELTCTASQKKSIQFHWKNSNQIKILGNQGSFLTKGPSKLNDRADSRRSLWDQGNFPLIIKNLKIEDSDTYICEVEDQKEEVQLLVFGLTANSDTHLLQGQSLTLTLESPPGSSPSVQCRSPRGKNIQGGKTLSVSQLELQDSGTWTCTVLQNQKKVEFKIDIVVLAFQKASSIVYKKEGEQVEFSFPLAFTVEKLTGSGELWWQAERASSSKSWITFDLKNKEVSVKRVTQDPKLQMGKKLPLHLTLPQALPQYAGSGNLTLALEAKTGKLHQEVNLVVMR

SEQ ID NO: 80 - DNA, 142 bp, Artificial Sequence
  synthetic
tgtttgcctgtgacatgaactcattgtgacacaaaccactgtgctaggggggatccactagtaacggccgccagtgtgctggaattcgccctcgcaagggccaggcatataagtacacaataaacaaatggcagctctctcc

SEQ ID NO: 81 - DNA, 99 bp, Artificial Sequence
  synthetic
cccctccttccttccccaggcactttccaagtgtcaactctagagcctatcgcggccgcaccggtataacttcgtataatgtatgctatacgaagttat

SEQ ID NO: 82 - DNA, 90 bp, Artificial Sequence
  synthetic
ataacttcgtataatgtatgctatacgaagttatgtcgacgtagcctatttctctagatccaaaatgatgacaacaaaaggtaccttgtg

SEQ ID NO: 83 - protein, 210 aa, Artificial Sequence
  synthetic
MQPWLWLVFSMKLAVLHGNSVLQQTPAYIKVQTNKMVMLSCEAKISLSNMRIYWLRQRQAPSSDSHHEFLALWDSAKGTIHGEEVEQEKIAVFRDASRFILNLTSVKPEDSGIYFCMIVGSPELTFGKGTQLSVVDFLPTTAQPTKKSTLKKRVCRLPRPETQKGLTCSLTTLSLLVVCILLLLAFLGVAVYFYCVRRRARIHFMKQFHK

SEQ ID NO: 84 - protein, 151 aa, Artificial Sequence
  synthetic
VLHGNSVLQQTPAYIKVQTNKMVMLSCEAKISLSNMRIYWLRQRQAPSSDSHHEFLALWDSAKGTIHGEEVEQEKIAVFRDASRFILNLTSVKPEDSGIYFCMIVGSPELTFGKGTQLSVVDFLPTTAQPTKKSTLKKRVCRLPRPETQKG

SEQ ID NO: 85 - DNA, 100 bp, Artificial Sequence
  synthetic
tgaacctgctgctgctgggtgagtcgattatcctggggagtggagaagctaggccgagccagttccgggtgtcgccgctggatcggacctggaacctggg

SEQ ID NO: 86 - DNA, 90 bp, Artificial Sequence
  synthetic
atgccagggacagccctgatactgtaggtagagtcaagggctgtccaagtaccggtataacttcgtataaggtatcctatacgaagttat

SEQ ID NO: 87 - DNA, 89 bp, Artificial Sequence
  synthetic
ataacttcgtataaggtatcctatacgaagttatctcgacctgatcttggagggagacctggaccgggagacgtgctgggggcagggtt

SEQ ID NO: 88 - protein, 243 aa, Artificial Sequence
  synthetic
MASPLTRFLSLNLLLLGESIILGSGEARPSQFRVSPLDRTWNLGETVELKCQVLLSNPTSGCSWLFQPRGAAASPTFLLYLSQNKPKAAEGLDTQRFSGKRLGDTFVLTLSDFRRENEGYYFCSALSNSIMYFSHFVPVFLPAKPTTTPAPRPPTPAPTIASQPLSLRPEACRPAAGGAVKGTGLDFACDIYIWAPLAGICVALLLSLIITLICYHRSRKRVCKCPRPLVRQEGKPRPSEKIV

SEQ ID NO: 89 - protein, 152 aa, Artificial Sequence
  synthetic
RPSQFRVSPLDRTWNLGETVELKCQVLLSNPTSGCSWLFQPRGAAASPTFLLYLSQNKPKAAEGLDTQRFSGKRLGDTFVLTLSDFRRENEGYYFCSALSNSIMYFSHFVPVFLPAKPTTTPAPRPPTPAPTIASQPLSLRPEACRPAAGGA

SEQ ID NO: 90 - DNA, 149 bp, Artificial Sequence
  Sequence of the chimeric human/mouse MHC I locus at the 5' junction of mouse/human sequences
agtgtcgccgcggacgctggatataaagtccacgcagcccgcagaactcagaagtcgcgaatcgccgacaggtgcgatggccgtcatggcgccccgaaccctcgtcctgctactctcgggggctctggccctgacccagacctgggcgg

SEQ ID NO: 91 - DNA, 159 bp, Artificial Sequence
  Sequence of the chimeric human/mouse MHC I locus at the 3' junction of human/mouse sequences
ggtggtgccttctggacaggagcagagatacacctgccatgtgcagcatgagggtttgcccaagcccctcaccctgagatggggtaaggagagtgtgggtgcagagctggggtcagggaaagctggagctttctgcagaccctgagctgctcagggctg